European Patent Application EP 4 215 208 A9, published August 30, 2023. Title: Pharmaceutical Combination and Use Thereof. Applicant: Shanghai Bao Pharmaceuticals Co., Ltd. The sequence listing filed with the application follows.

SEQUENCE LISTING (95 sequences)

SEQ ID NO: 1 - protein, 339 aa, Artificial Sequence
  IdeS
MRKRCYSTSAAVLAAVTLFVLSVDRGVIADSFSANQEIRYSEVTPYHVTSVWTKGVTPPANFTQGEDVFHAPYVANQGWYDITKTFNGKDDLLCGAATAGNMLHWWFDQNKDQIKRYLEEHPEKQKINFNGEQMFDVKEAIDTKNHQLDSKLFEYFKEKAFPYLSTKHLGVFPDHVIDMFINGYRLSLTNHGPTPVKEGSKDPRGGIFDAVFTRGDQSKLLTSRHDFKEKNLKEISDLIKKELTEGKALGLSHTYANVRINHVINLWGADFDSNGNLKAIYVTDSDSNASIGMKKYFVGVNSAGKVAISAKEIKEDNIGAQVLGLFTLSTGQDSWNQTN

SEQ ID NO: 2 - protein, 349 aa, Artificial Sequence
  IdeZ
MKTIAYPNKPHSLSAGLLTAIAIFSLASSNITYADDYQRNATEAYAKEVPHQITSVWTKGVTPLTPEQFRYNNEDVIHAPYLAHQGWYDITKAFDGKDNLLCGAATAGNMLHWWFDQNKTEIEAYLSKHPEKQKIIFNNQELFDLKAAIDTKDSQTNSQLFNYFRDKAFPNLSARQLGVMPDLVLDMFINGYYLNVFKTQSTDVNRPYQDKDKRGGIFDAVFTRGDQTTLLTARHDLKNKGLNDISTIIKQELTEGRALALSHTYANVSISHVINLWGADFNAEGNLEAIYVTDSDANASIGMKKYFVGINAHGHVAISAKKIEGENIGAQVLGLFTLSSGKDIWQKLS

SEQ ID NO: 3 - protein, 349 aa, Artificial Sequence
  IdeZ
MKTIAYPNKPHSLSAGLLTAIAIFSLASSNITYADDYQRNAAEVYAKEVPHQITSVWTKGVTPLTPEQFRYNNEDVIHAPYLAHQGWYDITKVFDGKDNLLCGAATAGNMLHWWFDQNKTEIEAYLSKHPEKQKIIFNNQELFDLKAAIDTKDSQTNSQLFNYFRDKAFPNLSARQLGVMPDLVLDMFINGYYLNVFKTQSTDVNRPYQDKDKRGGIFDAVFTRGDQTTLLTARHDLKNKGLNDISTIIKQELTEGRALALSHTYANVSISHVINLWGADFNAEGNLEAIYVTDSDANASIGMKKYFVGINAHGHVAISAKKIEGENIGAQVLGLFTLSSGKDIWQKLS

SEQ ID NO: 4 - protein, 392 aa, Artificial Sequence
  IdeZ2
MMKKQSFTHSRKPKFGMRKLSIGLASCMLGMMFLTTSHVSGEVVEVWPYGQDPNDKIEVLSQSEYSEYLQRLHDVEDFQAEKKKEGVVRTQWLEGVNVTDHDFRKITDGGSVYYATPLLNDRGYYDINKNFNQDSDKCAAAVAVNMFHYWLDRNKDNVAKFLSQSPDHGFVEGEPTFNLVDFQYTYASPYEEGGYRDNSKLFDFISKAFNKPLWANKLLDAYINGYGYIDRYVKNTPHSGQNNSKFNFFKKVFDGKLLTDIQQIFDYYTLSSELREALDTGKAIGLAYGPGDLRRSLGHIISVWGADINEDGNVVAIYVTDSDDKKLTIGNKKDRIGLKRYKLYSDNVGRARLTAYATENQQTGGEVRGIETLDMATQDWADYFSRTDEAEQ

SEQ ID NO: 5 - protein, 349 aa, Artificial Sequence
  IdeE
MKTIAYPNKPHSLSAGLLTAIAIFSLASSNITYADDYQRNATEAYAKEVPHQITSVWTKGVTPLTPEQFRYNNEDVIHAPYLAHQGWYDITKAFDGKDNLLCGAATAGNMLHWWFDQNKTEIEAYLSKHPEKQKIIFNNQELFDLKAAIDTKDSQTNSQLFNYFRDKAFPNLSARQLGVMPDLVLDMFINGYYLNVFKTQSTDVNRPYQDKDKRGGIFDAVFTRGDQTTLLTARHDLKNKGLNDISTIIKQELTEGRALALSHTYANVSISHVINLWGADFNAEGNLEAIYVTDSDANASIGMKKYFVGINAHRHVAISAKKIEGENIGAQVLGLFTLSSGKDIWQKLS

SEQ ID NO: 6 - protein, 385 aa, Artificial Sequence
  IdeE2
MMKKQSFTHSRKPKFGMRKLSIGLASCMLGMMFLTTGHVSGEVVEVWPNGQNPNGKIEILSQTEHSEHLQKLRDIEDFQAQKQADHVRYTKWLDGVTVDEHEFRKIKEYDTEYYVTPLLSGKGYYDINKDFNQDSDKCAAAVAANMFHYWFDRNRDSINRFLSQSPGENGVIKLENEKTIEVSKFLETYRSDGDYLDKSPFFDLISNSFKGPVWANKLLDAYINGYGYIHKFAKNTPHSKNNNSKFNFFKKVFDGNLLTDIHQIFDYNTFSDKLSEALYTGKAIGLAYGPGDLRRSLGHIISVWGADLDDQNRVVAIYVTDSDDKKLTIGNERVGLKRYKVSSDDQGRARLTTRDKDNTGGEIRSIETLDMGTQEWADYFNKTEK

SEQ ID NO: 7 - protein, 372 aa, Artificial Sequence
  IdeP
MNKKNSKGLPRYFRISARTLLLGALLSGGLLSVPEKAHADNRSASTISVSIDSNQNETNLVTAENVQTANLSDPDTKVNTVWTAGMSELDTKQFTPHPDGFLHYPYQSNQGWYNITKSFNGRDNLLCAAATAGNMLHWWFDQNKEQIDRYLKEHPEKANISFRGENFLSIKELINTKGKQKDSALFTYFQEKAFPDISRRNTGLIVDRVLDMFINGYYLSINDLSETNTSNTRKDNRGGVFDHVFGRGDSHKKLTSRYELQDQSIEEIGQLIRRELEAGKALAISYTYASIGMAHVVNLWGADFDQAGQLVAIYVADSDNSTDVGMKKYYVGKNKEGHVAISAQKVEGDVLGSRLLRLGSLSSGKDMWPAQY

SEQ ID NO: 8 - protein, 310 aa, Artificial Sequence
  pCART152
DSFSANQEIRYSEVTPYHVTSVWTKGVTPPANFTQGEDVFHAPYVANQGWYDITKTFNGKDDLLCGAATAGNMLHWWFDQNKDQIKRYLEEHPEKQKINFRGEQMFDVKEAIDTKNHQLDSKLFEYFKEKAFPYLSTKHLGVFPDHVIDMFINGYRLSLTNHGPTPVKEGSKDPRGGIFDAVFTRGDQSKLLTSRHDFKEKNLKEISDLIKKELTEGKALGLSHTYANVRINHVINLWGADFDSNGNLKAIYVTDSDSNASIGMKKYFVGVNSAGKVAISAKEIKEDNIGAQVLGLFTLSTGQDSWNQTN

SEQ ID NO: 9 - protein, 310 aa, Artificial Sequence
  pCART183
DSFSANQEIRYSEVTPYHVTSVWTKGVTPPANFTQGEDVFHAPYVANQGWYDITKTFNGKDDLLCGAATAGNMLHWWFDQNKDQIKRYLEEHPEKQKINFKGEQMFDVKEAIDTKNHQLDSKLFEYFKEKAFPYLSTKHLGVFPDHVIDMFINGYRLSLTNHGPTPVKRGSKDPRGGIFDAVFTRGNQSKLLTSRHDFKEKNLKEISDLIKKELTEGKALGLSHTYANVRINHVINLWGADFDSNGNLKAIYVTDSDSNASIGMKKYFVGVNSAGKVAISAKEIKEDNIGAQVLGLFTLSTGQDSWNQTN

SEQ ID NO: 10 - protein, 310 aa, Artificial Sequence
  pCART184
DSFSANQEIRYSEVTPYHVTSVWTKGVTPPANFTQGEDVFHAPYVANQGWYDITKTFNGKDDLLCGAATAGNMLHWWFDQNKDQIKRYLEEHPEKQKINFRGEQMFDVKEAIDTKNHQLDSKLFEYFKEKAFPYLSTKHLGVFPDHVIDMFINGYRLSLTNHGPTPVKKGSKDPRGGIFDAVFTRGNQSKLLTSRHDFKEKNLKEISDLIKKELTEGKALGLSHTYANVRINHVINLWGADFDSNGNLKAIYVTDSDSNASIGMKKYFVGVNKAGKVAISAKEIKEDNIGAQVLGLFTLSTGQDSWNQTN

SEQ ID NO: 11 - protein, 310 aa, Artificial Sequence
  pCART185
DSFSANQEIRYSEVTPYHVTSVWTKGVTPPANFTQGEDVFHAPYVANQGWYDITKTFNGKDDLLCGAATAGNMLHWWFDQNKDQIKRYLREHPEKQKINFNGEQMFDVKEAIDTKNHQLDSKLFEYFKEKAFPYLSTKHLGVFPDHVIDMFINGYRLSLTNHGPTPVKEGSKDPRGGIFDAVFTRGNQSKLLTSRHDFKEKNLKEISDLIKKELDEGKALGLSHTYANVRINHVINLWGADFDSNGNLKAIYVTDSDSNASIGMKKYFVGVNSAGKVAISAKEIKEDNIGAQVLGLFTLSTGQDSWNQTN

SEQ ID NO: 12 - protein, 310 aa, Artificial Sequence
  pCART186
DSFSANQEIRYSEVTPYHVTSVWTKGVTPPANFTQGEDVFHAPYVANQGWYDITKTFNGKDDLLCGAATAGNMLHWWFDQNKDQIKRYLKEHPEKQKINFNGEQMFDVKEAIRTKNHQLDSKLFEYFKEKAFPYLSTKHLGVFPDHVIDMFINGYRLSLTNHGPTPVKEGSKDPRGGIFDAVFTRGNQSKLLTSRHDFKEKNLKEISDLIKKELEEGKALGLSHTYANVRINHVINLWGADFDSNGNLKAIYVTDSDSNASIGMKKYFVGVNKAGKVAISAKEIKEDNIGAQVLGLFTLSTGQDSWNQTN

SEQ ID NO: 13 - protein, 310 aa, Artificial Sequence
  pCART187
DSFSANQEIRYSEVTPYHVTSVWTKGVTPPANFTQGEDVFHAPYVANQGWYDITKTFNGKDDLLCGAATAGNMLHWWFDQNKDQIERYLEEHPEKQKINFNGEQMFDVKEAIDTKNHQLDSKLFEYFKEKAFPYLSTKHLGVFPDHVIDMFINGYRLSLTNHGPTPVKEGSKDPRGGIFDAVFTRGNQSKLLTSRHDFKEKNLKEISDLIKEELTKGKALGLSHTYANVRINHVINLWGADFDSNGNLKAIYVTDSDSNASIGMKKYFVGVNSAGKVAISAKEIKEKNIGAQVLGLFTLSTGQKSWNQTN

SEQ ID NO: 14 - protein, 310 aa, Artificial Sequence
  pCART188
DSFSANQEIRYSEVTPYHVTSVWTKGVTPPANFTQGEDVFHAPYVANQGWYDITKTFNGKDDLLCGAATAGNMLHWWFDQNKDQIKRYLKEHPEKQKINFRGEQMFDVKEAIRTKNHQLDSKLFEYFKEKAFPYLSTKHLGVFPDHVIDMFINGYRLSLTNHGPTPVKEGSKDPRGGIFDAVFTRGNQSKLLTSRHDFKEKNLKEISDLIKSELENGKALGLSHTYANVRINHVINLWGADFDSNGNLKAIYVTDSDSNASIGMKKYFVGVNKAGKVAISAKEIKEDNIGAQVLGLFTLSTGQDSWNQTN

SEQ ID NO: 15 - protein, 310 aa, Artificial Sequence
  pCART189
DSFSANQEIRYSEVTPYHVTSVWTKGVTPPANFTQGEDVFHAPYVANQGWYDITKTFNGKDDLLCGAATAGNMLHWWFDQNKDQIKRYLKEHPEKQKINFRGEQMFDVKEAIRTKNHQLDSKLFEYFKEKAFPYLSTKHLGVFPDHVIDMFINGYRLSLTNHGPTPVKKGSKDPRGGIFDAVFTRGNQSKLLTSRHDFKEKNLKEISDLIKKELEEGKALGLSHTYANVRINHVINLWGADFDSNGNLKAIYVTDSDSNASIGMKKYFVGVNSAGKVAISAKEIKEDNIGAQVLGLFTLSTGQDSWNQTN

SEQ ID NO: 16 - protein, 310 aa, Artificial Sequence
  pCART190
DSFSANQEIRYSEVTPYHVTSVWTKGVTPPANFTQGEDVFHAPYVANQGWYDITKTFNGKDDLLCGAATAGNMLHWWFDQNKDQIERYLEEHPEKQKINFRGEQMFDVKEAIDTKNHQLDSKLFEYFKEKAFPYLSTKHLGVFPDHVIDMFINGYRLSLTNHGPTPVKKGSKDPRGGIFDAVFTRGNQSKLLTSRHDFKEKNLKEISDLIKEELTKGKALGLSHTYANVRINHVINLWGADFDSNGNLKAIYVTDSDSNASIGMKKYFVGVNSAGKVAISAKEIKEDNIGAQVLGLFTLSTGQKSWNQTN

SEQ ID NO: 17 - protein, 306 aa, Artificial Sequence
  pCART209
DSFSANQEIRYSEVTPYHVTSVWTKGVTPPANFTQGEDVFHAPYVANQGWYDITKTFNGKDDLLCGAATAGNMLHWWFDQNKDQIKRYLEEHPEKQKINFNGEQMFDVKEAIDTKNHQLDSKLFEYFKEKAFPYLSTKHLGVFPDHVIDMFINGYRLSLTNHGPTPVKEGSKDPRGGIFDAVFTRGDQSKLLTSRHDFKEKNLKEISDLIKKELTEGKALGLSHTYANVRINHVINLWGADFDSNGNLKAIYVTDSDSNASIGMKKYFVGVNSAGKVAISAKEIKEDNIGAQVLGLFTLSTGQDSW

SEQ ID NO: 18 - protein, 290 aa, Artificial Sequence
  pCART125
SVWTKGVTPPANFTQGEDVFHAPYVANQGWYDITKTFNGKDDLLCGAATAGNMLHWWFDQNKDQIKRYLEEHPEKQKINFNGEQMFDVKEAIDTKNHQLDSKLFEYFKEKAFPYLSTKHLGVFPDHVIDMFINGYRLSLTNHGPTPVKEGSKDPRGGIFDAVFTRGDQSKLLTSRHDFKEKNLKEISDLIKKELTEGKALGLSHTYANVRINHVINLWGADFDSNGNLKAIYVTDSDSNASIGMKKYFVGVNSAGKVAISAKEIKEDNIGAQVLGLFTLSTGQDSWNQTN

SEQ ID NO: 19 - protein, 290 aa, Artificial Sequence
  pCART213
SVWTKGVTPPANFTQGEDVFHAPYVANQGWYDITKTFNGKDDLLCGAATAGNMLHWWFDQNKDQIKRYLEEHPEKQKINFKGEQMFDVKEAIDTKNHQLDSKLFEYFKEKAFPYLSTKHLGVFPDHVIDMFINGYRLSLTNHGPTPVKEGSKDPRGGIFDAVFTRGNQSKLLTSRHDFKEKNLKEISDLIKKELTEGKALGLSHTYANVRINHVINLWGADFDSNGNLKAIYVTDSDSNASIGMKKYFVGVNSAGKVAISAKEIKEDNIGAQVLGLFTLSTGQDSWNQTN

SEQ ID NO: 20 - protein, 290 aa, Artificial Sequence
  pCART214
SVWTKGVTPPANFTQGEDVFHAPYVANQGWYDITKTFNGKDDLLCGAATAGNMLHWWFDQNKDQIERYLEEHPEKQKINFKGEQMFDVKKAIDTKNHQLDSKLFEYFKEKAFPYLSTKHLGVFPDHVIDMFINGYRLSLTNHGPTPVKEGSKDPRGGIFDAVFTRGNQSKLLTSRHDFKEKNLKEISDLIKEELTKGKALGLSHTYANVRINHVINLWGADFDSNGNLKAIYVTDSDSNASIGMKKYFVGVNSAGKVAISAKEIKEDNIGAQVLGLFTLSTGQKSWNQTN

SEQ ID NO: 21 - protein, 319 aa, Artificial Sequence
  pCART228
DDYQRNATEAYAKEVPHQITSVWTKGVTPPANFTQGEDVFHAPYVANQGWYDITKTFNGKDDLLCGAATAGNMLHWWFDQNKDQIERYLEEHPEKQKINFKGEQMFDVKKAIDTKNHQLDSKLFEYFKEKAFPYLSTKHLGVFPDHVIDMFINGYRLSLTNHGPTPVKEGSKDPRGGIFDAVFTRGNQSKLLTSRHDFKEKNLKEISDLIKEELTKGKALGLSHTYANVRINHVINLWGADFDSNGNLKAIYVTDSDSNASIGMKKYFVGVNSAGKVAISAKEIKEDNIGAQVLGLFTLSTGQKSWNQTNGGGHHHHHH

SEQ ID NO: 22 - protein, 313 aa, Artificial Sequence
  Sequence of hybrid IdeS/Z
DDYQRNATEAYAKEVPHQITSVWTKGVTPLTPEQFRYNNEDVFHAPYVANQGWYDITKAFDGKDNLLCGAATAGNMLHWWFDQNKDQIKRYLEEHPEKQKINFNGDNMFDVKKAIDTKNHQLDSKLFNYFKEKAFPGLSARRIGVFPDHVIDMFINGYRLSLTNHGPTPVKEGSKDPRGGIFDAVFTRGNQSKLLTSRHDFKNKNLNDISTIIKQELTKGKALGLSHTYANVSINHVINLWGADFNAEGNLEAIYVTDSDSNASIGMKKYFVGVNAHGHVAISAKKIEGENIGAQVLGLFTLSTGQDSWQKLS

SEQ ID NO: 23 - protein, 315 aa, Artificial Sequence
  pCART197
DDYQRNATEAYAKEVPHQITSVWTKGVTPLTPEQFRYNNEDVIHAPYLANQGWYDITKAFDGKDNLLCGAATAGNMLHWWFDQNKTEIEAYLSKHPEKQKIIFRNQELFDLKEAIRTKDSQTNSQLFEYFRDKAFPYLSARQLGVMPDLVLDMFINGYYLNVFKTQSTDVKRPYQDKDKRGGIFDAVFTRGNQTTLLTARHDLKNKGLNDISTIIKEELTKGRALALSHTYANVSISHVINLWGADFNAEGNLEAIYVTDSDANASIGMKKYFVGINKHGHVAISAKKIEGENIGAQVLGLFTLSSGKDIWQKLN

SEQ ID NO: 24 - protein, 315 aa, Artificial Sequence
  pCART198
DDYQRNATEAYAKEVPHQITSVWTKGVTPLTPEQFRYNNEDVIHAPYLAHQGWYDITKTFNGKDNLLCGAATAGNMLHWWFDQNKTEIEAYLSKHPEKQKIIFNNEELFDLKAAIDTKDSQTNSQLFNYFKEKAFPNLSTRQLGVMPDLVLDMFINGYYLNVFKTQSTDVNRPYQDKDKRGGIFDAVFTRGNQTTLLTARHDFKEKGLKDISTIIKQELTEGRALALSHTYANVSISHVINLWGADFDAEGNLKAIYVTDSDANASIGMKKYFVGINAHGKVAISAKKIEGENIGAQVLGLFTLSSGKDIWQQLS

SEQ ID NO: 25 - protein, 315 aa, Artificial Sequence
  pCART200
DSFSANQEIRYSEVTPYHVTSVWTKGVTPLTPEQFRYNNEDVIHAPYLAHQGWYDITKAFDGKDNLLCGAATAGNMLHWWFDQNKTEIEAYLSKHPEKQKIIFNNQELFDLKAAIDTKDSQTNSQLFNYFRDKAFPNLSARQLGVMPDLVLDMFINGYYLNVFKTQSTDVNRPYQDKDKRGGIFDAVFTRGDQTTLLTARHDLKNKGLNDISTIIKQELTEGRALALSHTYANVSISHVINLWGADFNAEGNLEAIYVTDSDANASIGMKKYFVGINAHGHVAISAKKIEGENIGAQVLGLFTLSSGKDIWQKLS

SEQ ID NO: 26 - protein, 295 aa, Artificial Sequence
  pCART201
SVWTKGVTPLTPEQFRYNNEDVIHAPYLAHQGWYDITKAFDGKDNLLCGAATAGNMLHWWFDQNKTEIEAYLSKHPEKQKIIFNNQELFDLKAAIDTKDSQTNSQLFNYFRDKAFPNLSARQLGVMPDLVLDMFINGYYLNVFKTQSTDVNRPYQDKDKRGGIFDAVFTRGDQTTLLTARHDLKNKGLNDISTIIKQELTEGRALALSHTYANVSISHVINLWGADFNAEGNLEAIYVTDSDANASIGMKKYFVGINAHGHVAISAKKIEGENIGAQVLGLFTLSSGKDIWQKLS

SEQ ID NO: 27 - protein, 314 aa, Artificial Sequence
  pCART202
DDYQRNATEAYAKEVPHQITSVWTKGVTPLTPEQFTQGEDVIHAPYLAHQGWYDITKAFDGKDNLLCGAATAGNMLHWWFDQNKTEIEAYLSKHPEKQKIIFNNQELFDLKAAIDTKDSQTNSQLFNYFRDKAFPNLSARQLGVMPDLVLDMFINGYYLNVFKTQSTDVNRPYQDKDKRGGIFDAVFTRGDQTTLLTARHDLKNKGLNDISTIIKQELTEGRALALSHTYANVSISHVINLWGADFNAEGNLEAIYVTDSDANASIGMKKYFVGINAHGHVAISAKKIEGENIGAQVLGLFTLSSGKDIWQKLS

SEQ ID NO: 28 - protein, 312 aa, Artificial Sequence
  pCART203
DDYQRNATEAYAKEVPHQITSVWTKGVTPPEQFTQGEDVIHAPYLAHQGWYDITKAFDGKDNLLCGAATAGNMLHWWFDQNKTEIEAYLSKHPEKQKIIFNNQELFDLKAAIDTKDSQTNSQLFNYFRDKAFPNLSARQLGVMPDLVLDMFINGYYLNVFKTQSTDVNRPYQDKDKRGGIFDAVFTRGDQTTLLTARHDLKNKGLNDISTIIKQELTEGRALALSHTYANVSISHVINLWGADFNAEGNLEAIYVTDSDANASIGMKKYFVGINAHGHVAISAKKIEGENIGAQVLGLFTLSSGKDIWQKLS

SEQ ID NO: 29 - protein, 313 aa, Artificial Sequence
  pCART204
DDYQRNATEAYAKEVPHQITSVWTKGVTPPEQFRYNNEDVIHAPYLAHQGWYDITKAFDGKDNLLCGAATAGNMLHWWFDQNKTEIEAYLSKHPEKQKIIFNNQELFDLKAAIDTKDSQTNSQLFNYFRDKAFPNLSARQLGVMPDLVLDMFINGYYLNVFKTQSTDVNRPYQDKDKRGGIFDAVFTRGDQTTLLTARHDLKNKGLNDISTIIKQELTEGRALALSHTYANVSISHVINLWGADFNAEGNLEAIYVTDSDANASIGMKKYFVGINAHGHVAISAKKIEGENIGAQVLGLFTLSSGKDIWQKLS

SEQ ID NO: 30 - protein, 312 aa, Artificial Sequence
  pCART 206
DDYQRNATEAYAKEVPHQITSVWTKGVTPPEQFTQGEDVIHAPYLAHQGWYDITKAFDGKDNLLCGAATAGNMLHWWFDQNKTEIEAYLSKHPEKQKIIINNQELFDLKAAIDTKDSQTNSQLFNYFRDKAFPNLSARQLGVMPDLVLDMFINGYYLNVFKTQSTDVNRPYQDKDKRGGIFDAVFTRGDQTTLLTARHDLKNKGLNDISTIIKQELTEGRALALSHTYANVSISHVINLWGADFNAEGNLEAIYVTDSDANASIGMKKYFVGINAHGHVAISAKKIEGENIGAQVLGLFTLSSGKDIWQKLS

SEQ ID NO: 31 - protein, 312 aa, Artificial Sequence
  pCART207
DDYQRNATEAYAKEVPHQITSVWTKGVTPPEQFTQGEDVIHAPYLAHQGWYDITKAFDGKDNLLCGAATAGNMLHWWFDQNKTEIEAYLSKHPEKQKIIFRNQELFDLKAAIDTKDSQTNSQLFNYFRDKAFPNLSARQLGVMPDLVLDMFINGYYLNVFKTQSTDVNRPYQDKDKRGGIFDAVFTRGDQTTLLTARHDLKNKGLNDISTIIKQELTEGRALALSHTYANVSISHVINLWGADFNAEGNLEAIYVTDSDANASIGMKKYFVGINAHGHVAISAKKIEGENIGAQVLGLFTLSSGKDIWQKLS

SEQ ID NO: 32 - protein, 312 aa, Artificial Sequence
  pCART208
DDYQRNATEAYAKEVPHQITSVWTKGVTPPEQFTQGEDVIHAPYLAHQGWYDITKAFDGKDNLLCGAATAGNMLHWWFDQNKTEIEAYLSKHPEKQKIIIRNQELFDLKAAIDTKDSQTNSQLFNYFRDKAFPNLSARQLGVMPDLVLDMFINGYYLNVFKTQSTDVNRPYQDKDKRGGIFDAVFTRGDQTTLLTARHDLKNKGLNDISTIIKQELTEGRALALSHTYANVSISHVINLWGADFNAEGNLEAIYVTDSDANASIGMKKYFVGINAHGHVAISAKKIEGENIGAQVLGLFTLSSGKDIWQKLS

SEQ ID NO: 33 - protein, 312 aa, Artificial Sequence
  pCART210
DDYQRNATEAYAKEVPHQITSVWTKGVTPPEQFTQGEDVIHAPYLANQGWYDITKAFDGKDNLLCGAATAGNMLHWWFDQNKTEIEAYLSKHPEKQKIIFRNQELFDLKEAIRTKDSQTNSQLFEYFRDKAFPYLSARQLGVMPDLVLDMFINGYYLNVFKTQSTDVKRPYQDKDKRGGIFDAVFTRGNQTTLLTARHDLKNKGLNDISTIIKEELTKGRALALSHTYANVSISHVINLWGADFNAEGNLEAIYVTDSDANASIGMKKYFVGINKHGHVAISAKKIEGENIGAQVLGLFTLSSGKDIWQKLN

SEQ ID NO: 34 - protein, 292 aa, Artificial Sequence
  pCART217
SVWTKGVTPPEQFTQGEDVIHAPYLAHQGWYDITKAFDGKDNLLCGAATAGNMLHWWFDQNKTEIEAYLSKHPEKQKIIFRNQELFDLKAAIDTKDSQTNSQLFNYFRDKAFPNLSARQLGVMPDLVLDMFINGYYLNVFKTQSTDVNRPYQDKDKRGGIFDAVFTRGNQTTLLTARHDLKNKGLNDISTIIKQELTEGRALALSHTYANVSISHVINLWGADFNAEGNLEAIYVTDSDANASIGMKKYFVGINAHGHVAISAKKIEGENIGAQVLGLFTLSSGKDIWQKLS

SEQ ID NO: 35 - protein, 312 aa, Artificial Sequence
  pCART219
DDYQRNATEAYAKEVPHQITSVWTKGVTPPEQFTQGEDVIHAPYLAHQGWYDITKAFDGADNLLCGAATAGNMLHWWFDQNKTEIEAYLSKHPEKQKIIFRNQELFDLKAAIDTKDSQTNSQLFNYFRDKAFPNLSARQLGVMPDLVLDMFINGYYLNVFKTQSTDVNRPYQDKDKRGGIFDAVFTRGNQTTLLTARHDLKNKGLNDISTIIKQELTEGRALALSHTYANVSISHVINLWGADFNAEGNLEAIYVTDSDANASIGMKKYFVGINAHGHVAISAKKIEGENIGAQVLGLFTLSSGKDIWQKLS

SEQ ID NO: 36 - protein, 292 aa, Artificial Sequence
  pCART226
SVWTKGVTPPEQFTQGEDVIHAPYLAHQGWYDITKAFDGADNLLCGAATAGNMLHWWFDQNKTEIEAYLSKHPEKQKIIFRNQELFDLKAAIDTKDSQTNSQLFNYFRDKAFPNLSARQLGVMPDLVLDMFINGYYLNVFKTQSTDVNRPYQDKDKRGGIFDAVFTRGNQTTLLTARHDLKNKGLNDISTIIKQELTEGRALALSHTYANVSISHVINLWGADFNAEGNLEAIYVTDSDANASIGMKKYFVGINAHGHVAISAKKIEGENIGAQVLGLFTLSSGKDIWQKLS

SEQ ID NO: 37 - protein, 312 aa, Artificial Sequence
  pCART229
DDYQRNATEAYAKEVPHQITSVWTKGVTPPEQFTQGEDVIHAPYLAHQGWYDITKAFDGKDNLLCGAATAGNMLHWWFDQNKTEIEAYLSKHPEKQKIIFRNQELFDLKAAIDTKDSQTNSQLFNYFRDKAFPNLSARQLGVMPDLVLDMFINGYYLNVFKTQSTDVNRPYQDKDKRGGIFDAVFTRGNQTTLLTARHDLKNKGLNDISTIIKQELTEGRALALSHTYANVSISHVINLWGADFNAEGNLEAIYVTDSDANASIGMKKYFVGINAHGHVAISAKKIEGENIGAQVLGLFTLSSGKDIWQKLS

SEQ ID NO: 38 - protein, 312 aa, Artificial Sequence
  pCARTI91
DDYQRNATEAYAKEVPHQITSVWTKGVTPLTPEQFTQGEDVFHAPYVANQGWYDITKAFDGKDNLLCGAATAGNMLHWWFDQNKDQIKRYLEEHPEKQKINFNGENMFDVKKAIDTKNHQLDSKLFNYFKEKAFPYLSAKHLGVFPDHVIDMFINGYRLSLTNHGPTPVKEGSKDPRGGIFDAVFTRGNQSKLLTSRHDFKNKNLNDISTIIKQELTKGKALGLSHTYANVRINHVINLWGADFNAEGNLEAIYVTDSDSNASIGMKKYFVGVNAHGHVAISAKKIEGENIGAQVLGLFTLSTGQDSWQKLS

SEQ ID NO: 39 - protein, 312 aa, Artificial Sequence
  pCART192
DDYQRNATEAYAKEVPHQITSVWTKGVTPLTPEQFTQGEDVFHAPYVANQGWYDITKAFDGKDNLLCGAATAGNMLHWWFDQNKDQIKRYLEEHPEKQKINFRGENMFDVKEAIRTKNHQLDSKLFEYFKEKAFPYLSAKHLGVFPDHVIDMFINGYRLSLTNHGPTPVKKGSKDPRGGIFDAVFTRGNQSKLLTSRHDFKNKNLNDISTIIKSELTNGKALGLSHTYANVRINHVINLWGADFNAEGNLEAIYVTDSDSNASIGMKKYFVGVNKHGHVAISAKKIEGENIGAQVLGLFTLSTGQDSWQKLN

SEQ ID NO: 40 - protein, 312 aa, Artificial Sequence
  pCARTI93
DDYQRNATEAYAKEVPHQITSVWTKGVTPLTPEQFTQGEDVFHAPYVANQGWYDITKTFNGKDDLLCGAATAGNMLHWWFDQNKDQIKRYLEEHPEKQKINFNGEQMFDVKEAIDTKNHQLDSKLFEYFKEKAFPYLSTKHLGVFPDHVIDMFINGYRLSLTNHGPTPVKEGSKDPRGGIFDAVFTRGNQSKLLTSRHDFKEKNLKEISDLIKQELTEGKALGLSHTYANVRINHVINLWGADFDAEGNLKAIYVTDSDSNASIGMKKYFVGVNAAGKVAISAKKIEGENIGAQVLGLFTLSTGQDSWNQTS

SEQ ID NO: 41 - protein, 312 aa, Artificial Sequence
  pCART194
DDYQRNATEAYAKEVPHQITSVWTKGVTPLTPEQFTQGEDVFHAPYVANQGWYDITKTFNGKDDLLCGAATAGNMLHWWFDQNKDQIKRYLEEHPEKQKINFRGEQMFDVKEAIRTKNHQLDSKLFEYFKEKAFPYLSTKHLGVFPDHVIDMFINGYRLSLTNHGPTPVKKGSKDPRGGIFDAVFTRGNQSKLLTSRHDFKEKNLKEISDLIKEELTKGKALGLSHTYANVRINHVINLWGADFDAEGNLKAIYVTDSDSNASIGMKKYFVGVNKAGKVAISAKKIEGENIGAQVLGLFTLSTGQDSWNQTN

SEQ ID NO: 42 - protein, 310 aa, Artificial Sequence
  pCART205
DDYQRNATEAYAKEVPHQITSVWTKGVTPPEQFTQGEDVIHAPYVANQGWYDITKAFDGKDNLLCGAATAGNMLHWWFDQNKDQIKRYLEEHPEKQKINFRGEQMFDVKKAIDTKNHQLDSKLFNYFKEKAFPGLSARRIGVFPDHVIDMFINGYRLSLTNHGPTPVKEGSKDPRGGIFDAVFTRGNQSKLLTSRHDFKNKNLNDISTIIKQELTKGKALGLSHTYANVSINHVINLWGADFNAEGNLEAIYVTDSDSNASIGMKKYFVGVNAHGHVAISAKKIEGENIGAQVLGLFTLSTGQDSWQKLS

SEQ ID NO: 43 - protein, 11 aa, Artificial Sequence
  Light chain CDR1
RASQSVSSYLA

SEQ ID NO: 44 - protein, 7 aa, Artificial Sequence
  Light chain CDR2
DASNRAT

SEQ ID NO: 45 - protein, 10 aa, Artificial Sequence
  Light chain CDR3
QQRSNWPPTF

SEQ ID NO: 46 - protein, 5 aa, Artificial Sequence
  Heavy chain CDR1
SFAMS

SEQ ID NO: 47 - protein, 17 aa, Artificial Sequence
  Heavy chain CDR2
AISGSGGGTYYADSVKG

SEQ ID NO: 48 - protein, 13 aa, Artificial Sequence
  Heavy chain CDR3
DKILWFGEPVFDY

SEQ ID NO: 49 - protein, 11 aa, Artificial Sequence
  Light chain CDR1
KASQDVSTVVA

SEQ ID NO: 50 - protein, 7 aa, Artificial Sequence
  Light chain CDR2
SASYRYI

SEQ ID NO: 51 - protein, 9 aa, Artificial Sequence
  Light chain CDR3
QQHYSPPYT

SEQ ID NO: 52 - protein, 5 aa, Artificial Sequence
  Heavy chain CDR1
DYWMQ

SEQ ID NO: 53 - protein, 17 aa, Artificial Sequence
  Heavy chain CDR2
TIYPGDGDTGYAQKFQG

SEQ ID NO: 54 - protein, 11 aa, Artificial Sequence
  Heavy chain CDR3
GDYYGSNSLDY

SEQ ID NO: 55 - protein, 107 aa, Artificial Sequence [sequence omitted]

SEQ ID NO: 56 - protein, 124 aa, Artificial Sequence
  Heavy chain variable region
EVQLLESGGGLVQPGGSLRLSCAVSGFTFNSFAMSWVRQAPGKGLEWVSAISGSGGGTYYADSVKGRFTISRDNSKNTLYLQMNSLRAEDTAVYFCAKDKILWFGEPVFDYWGQGTLVTVSSAS

SEQ ID NO: 57 - protein, 108 aa, Artificial Sequence
  Light chain variable region
DIVMTQSHLSMSTSLGDPVSITCKASQDVSTVVAWYQQKPGQSPRRLIYSASYRYIGVPDRFTGSGAGTDFTFTISSVQAEDLAVYYCQQHYSPPYTFGGGTKLEIKR

SEQ ID NO: 58 - protein, 94 aa, Artificial Sequence
  Heavy chain variable region
QVQLVQSGAEVAKPGTSVKLSCKASGYTFTDYWMQWVKQRPGQGLEWIGTIYPGDGDTGYAQKFQGKATLTADKSSKTVYMHLSSLASEDSAVY

SEQ ID NO: 59 - protein, 173 aa, Artificial Sequence
  MMP3
FRTFPGIPKWRKTHLTYRIVNYTPDLPKDAVDSAVEKALKVWEEVTPLTFSRLYEGEADIMISFAVREHGDFYPFDGPGNVLAHAYAPGPGINGDAHFDDDEQWTKDTTGTNLFLVAAHEIGHSLGLFHSANTEALMYPLYHSLTDLTRFRLSQDDINGIQSLYGPPPDSPET

SEQ ID NO: 60 - protein, 172 aa, Artificial Sequence
  MMP12
FREMPGGPVWRKHYITYRINNYTPDMNREDVDYAIRKAFQVWSNVTPLKFSKINTGMADILVVFARGAHGDFHAFDGKGGILAHAFGPGSGIGGDAHFDEDEFWTTHSGGTNLFLTAVHEIGHSLGLGHSSDPKAVMFPTYKYVDINTFRLSADDIRGIQSLYGDPKENQRL

SEQ ID NO: 61 - protein, 349 aa, Artificial Sequence; identical to SEQ ID NO: 5
  IdeE complete sequence

SEQ ID NO: 62 - protein, 315 aa, Artificial Sequence
  IdeE sequence
DDYQRNATEAYAKEVPHQITSVWTKGVTPLTPEQFRYNNEDVIHAPYLAHQGWYDITKAFDGKDNLLCGAATAGNMLHWWFDQNKTEIEAYLSKHPEKQKIIFNNQELFDLKAAIDTKDSQTNSQLFNYFRDKAFPNLSARQLGVMPDLVLDMFINGYYLNVFKTQSTDVNRPYQDKDKRGGIFDAVFTRGDQTTLLTARHDLKNKGLNDISTIIKQELTEGRALALSHTYANVSISHVINLWGADFNAEGNLEAIYVTDSDANASIGMKKYFVGINAHRHVAISAKKIEGENIGAQVLGLFTLSSGKDIWQKLS

SEQ ID NO: 63 - protein, 315 aa, Artificial Sequence
  T8D
DDYQRNADEAYAKEVPHQITSVWTKGVTPLTPEQFRYNNEDVIHAPYLAHQGWYDITKAFDGKDNLLCGAATAGNMLHWWFDQNKTEIEAYLSKHPEKQKIIFNNQELFDLKAAIDTKDSQTNSQLFNYFRDKAFPNLSARQLGVMPDLVLDMFINGYYLNVFKTQSTDVNRPYQDKDKRGGIFDAVFTRGDQTTLLTARHDLKNKGLNDISTIIKQELTEGRALALSHTYANVSISHVINLWGADFNAEGNLEAIYVTDSDANASIGMKKYFVGINAHRHVAISAKKIEGENIGAQVLGLFTLSSGKDIWQKLS

SEQ ID NO: 64 - protein, 315 aa, Artificial Sequence
  T8E
DDYQRNAEEAYAKEVPHQITSVWTKGVTPLTPEQFRYNNEDVIHAPYLAHQGWYDITKAFDGKDNLLCGAATAGNMLHWWFDQNKTEIEAYLSKHPEKQKIIFNNQELFDLKAAIDTKDSQTNSQLFNYFRDKAFPNLSARQLGVMPDLVLDMFINGYYLNVFKTQSTDVNRPYQDKDKRGGIFDAVFTRGDQTTLLTARHDLKNKGLNDISTIIKQELTEGRALALSHTYANVSISHVINLWGADFNAEGNLEAIYVTDSDANASIGMKKYFVGINAHRHVAISAKKIEGENIGAQVLGLFTLSSGKDIWQKLS

SEQ ID NO: 65 - protein, 315 aa, Artificial Sequence
  T8W
DDYQRNAWEAYAKEVPHQITSVWTKGVTPLTPEQFRYNNEDVIHAPYLAHQGWYDITKAFDGKDNLLCGAATAGNMLHWWFDQNKTEIEAYLSKHPEKQKIIFNNQELFDLKAAIDTKDSQTNSQLFNYFRDKAFPNLSARQLGVMPDLVLDMFINGYYLNVFKTQSTDVNRPYQDKDKRGGIFDAVFTRGDQTTLLTARHDLKNKGLNDISTIIKQELTEGRALALSHTYANVSISHVINLWGADFNAEGNLEAIYVTDSDANASIGMKKYFVGINAHRHVAISAKKIEGENIGAQVLGLFTLSSGKDIWQKLS

SEQ ID NO: 66 - protein, 315 aa, Artificial Sequence
  T8Y
DDYQRNAYEAYAKEVPHQITSVWTKGVTPLTPEQFRYNNEDVIHAPYLAHQGWYDITKAFDGKDNLLCGAATAGNMLHWWFDQNKTEIEAYLSKHPEKQKIIFNNQELFDLKAAIDTKDSQTNSQLFNYFRDKAFPNLSARQLGVMPDLVLDMFINGYYLNVFKTQSTDVNRPYQDKDKRGGIFDAVFTRGDQTTLLTARHDLKNKGLNDISTIIKQELTEGRALALSHTYANVSISHVINLWGADFNAEGNLEAIYVTDSDANASIGMKKYFVGINAHRHVAISAKKIEGENIGAQVLGLFTLSSGKDIWQKLS

SEQ ID NO: 67 - protein, 315 aa, Artificial Sequence
  A10K
DDYQRNATEKYAKEVPHQITSVWTKGVTPLTPEQFRYNNEDVIHAPYLAHQGWYDITKAFDGKDNLLCGAATAGNMLHWWFDQNKTEIEAYLSKHPEKQKIIFNNQELFDLKAAIDTKDSQTNSQLFNYFRDKAFPNLSARQLGVMPDLVLDMFINGYYLNVFKTQSTDVNRPYQDKDKRGGIFDAVFTRGDQTTLLTARHDLKNKGLNDISTIIKQELTEGRALALSHTYANVSISHVINLWGADFNAEGNLEAIYVTDSDANASIGMKKYFVGINAHRHVAISAKKIEGENIGAQVLGLFTLSSGKDIWQKLS

SEQ ID NO: 68 - protein, 315 aa, Artificial Sequence
  A10R
DDYQRNATERYAKEVPHQITSVWTKGVTPLTPEQFRYNNEDVIHAPYLAHQGWYDITKAFDGKDNLLCGAATAGNMLHWWFDQNKTEIEAYLSKHPEKQKIIFNNQELFDLKAAIDTKDSQTNSQLFNYFRDKAFPNLSARQLGVMPDLVLDMFINGYYLNVFKTQSTDVNRPYQDKDKRGGIFDAVFTRGDQTTLLTARHDLKNKGLNDISTIIKQELTEGRALALSHTYANVSISHVINLWGADFNAEGNLEAIYVTDSDANASIGMKKYFVGINAHRHVAISAKKIEGENIGAQVLGLFTLSSGKDIWQKLS

SEQ ID NO: 69 - protein, 315 aa, Artificial Sequence
  T24A
DDYQRNATEAYAKEVPHQITSVWAKGVTPLTPEQFRYNNEDVIHAPYLAHQGWYDITKAFDGKDNLLCGAATAGNMLHWWFDQNKTEIEAYLSKHPEKQKIIFNNQELFDLKAAIDTKDSQTNSQLFNYFRDKAFPNLSARQLGVMPDLVLDMFINGYYLNVFKTQSTDVNRPYQDKDKRGGIFDAVFTRGDQTTLLTARHDLKNKGLNDISTIIKQELTEGRALALSHTYANVSISHVINLWGADFNAEGNLEAIYVTDSDANASIGMKKYFVGINAHRHVAISAKKIEGENIGAQVLGLFTLSSGKDIWQKLS

SEQ ID NO: 70 - protein, 315 aa, Artificial Sequence
  T24G
DDYQRNATEAYAKEVPHQITSVWGKGVTPLTPEQFRYNNEDVIHAPYLAHQGWYDITKAFDGKDNLLCGAATAGNMLHWWFDQNKTEIEAYLSKHPEKQKIIFNNQELFDLKAAIDTKDSQTNSQLFNYFRDKAFPNLSARQLGVMPDLVLDMFINGYYLNVFKTQSTDVNRPYQDKDKRGGIFDAVFTRGDQTTLLTARHDLKNKGLNDISTIIKQELTEGRALALSHTYANVSISHVINLWGADFNAEGNLEAIYVTDSDANASIGMKKYFVGINAHRHVAISAKKIEGENIGAQVLGLFTLSSGKDIWQKLS

SEQ ID NO: 71 - protein, 315 aa, Artificial Sequence
  T24S
DDYQRNATEAYAKEVPHQITSVWSKGVTPLTPEQFRYNNEDVIHAPYLAHQGWYDITKAFDGKDNLLCGAATAGNMLHWWFDQNKTEIEAYLSKHPEKQKIIFNNQELFDLKAAIDTKDSQTNSQLFNYFRDKAFPNLSARQLGVMPDLVLDMFINGYYLNVFKTQSTDVNRPYQDKDKRGGIFDAVFTRGDQTTLLTARHDLKNKGLNDISTIIKQELTEGRALALSHTYANVSISHVINLWGADFNAEGNLEAIYVTDSDANASIGMKKYFVGINAHRHVAISAKKIEGENIGAQVLGLFTLSSGKDIWQKLS

SEQ ID NO: 72 - protein, 315 aa, Artificial Sequence
  A59I
DDYQRNATEAYAKEVPHQITSVWTKGVTPLTPEQFRYNNEDVIHAPYLAHQGWYDITKIFDGKDNLLCGAATAGNMLHWWFDQNKTEIEAYLSKHPEKQKIIFNNQELFDLKAAIDTKDSQTNSQLFNYFRDKAFPNLSARQLGVMPDLVLDMFINGYYLNVFKTQSTDVNRPYQDKDKRGGIFDAVFTRGDQTTLLTARHDLKNKGLNDISTIIKQELTEGRALALSHTYANVSISHVINLWGADFNAEGNLEAIYVTDSDANASIGMKKYFVGINAHRHVAISAKKIEGENIGAQVLGLFTLSSGKDIWQKLS

SEQ ID NO: 73 - protein, 315 aa, Artificial Sequence
  A59L
DDYQRNATEAYAKEVPHQITSVWTKGVTPLTPEQFRYNNEDVIHAPYLAHQGWYDITKLFDGKDNLLCGAATAGNMLHWWFDQNKTEIEAYLSKHPEKQKIIFNNQELFDLKAAIDTKDSQTNSQLFNYFRDKAFPNLSARQLGVMPDLVLDMFINGYYLNVFKTQSTDVNRPYQDKDKRGGIFDAVFTRGDQTTLLTARHDLKNKGLNDISTIIKQELTEGRALALSHTYANVSISHVINLWGADFNAEGNLEAIYVTDSDANASIGMKKYFVGINAHRHVAISAKKIEGENIGAQVLGLFTLSSGKDIWQKLS

SEQ ID NO: 74 - protein, 315 aa, Artificial Sequence
  A59V
DDYQRNATEAYAKEVPHQITSVWTKGVTPLTPEQFRYNNEDVIHAPYLAHQGWYDITKVFDGKDNLLCGAATAGNMLHWWFDQNKTEIEAYLSKHPEKQKIIFNNQELFDLKAAIDTKDSQTNSQLFNYFRDKAFPNLSARQLGVMPDLVLDMFINGYYLNVFKTQSTDVNRPYQDKDKRGGIFDAVFTRGDQTTLLTARHDLKNKGLNDISTIIKQELTEGRALALSHTYANVSISHVINLWGADFNAEGNLEAIYVTDSDANASIGMKKYFVGINAHRHVAISAKKIEGENIGAQVLGLFTLSSGKDIWQKLS

SEQ ID NO: 75 - protein, 315 aa, Artificial Sequence
  E97D
DDYQRNATEAYAKEVPHQITSVWTKGVTPLTPEQFRYNNEDVIHAPYLAHQGWYDITKAFDGKDNLLCGAATAGNMLHWWFDQNKTEIEAYLSKHPDKQKIIFNNQELFDLKAAIDTKDSQTNSQLFNYFRDKAFPNLSARQLGVMPDLVLDMFINGYYLNVFKTQSTDVNRPYQDKDKRGGIFDAVFTRGDQTTLLTARHDLKNKGLNDISTIIKQELTEGRALALSHTYANVSISHVINLWGADFNAEGNLEAIYVTDSDANASIGMKKYFVGINAHRHVAISAKKIEGENIGAQVLGLFTLSSGKDIWQKLS

SEQ ID NO: 76 - protein, 315 aa, Artificial Sequence
  R280H
DDYQRNATEAYAKEVPHQITSVWTKGVTPLTPEQFRYNNEDVIHAPYLAHQGWYDITKAFDGKDNLLCGAATAGNMLHWWFDQNKTEIEAYLSKHPEKQKIIFNNQELFDLKAAIDTKDSQTNSQLFNYFRDKAFPNLSARQLGVMPDLVLDMFINGYYLNVFKTQSTDVNRPYQDKDKRGGIFDAVFTRGDQTTLLTARHDLKNKGLNDISTIIKQELTEGRALALSHTYANVSISHVINLWGADFNAEGNLEAIYVTDSDANASIGMKKYFVGINAHHHVAISAKKIEGENIGAQVLGLFTLSSGKDIWQKLS

SEQ ID NO: 77 - protein, 315 aa, Artificial Sequence
  R280K
DDYQRNATEAYAKEVPHQITSVWTKGVTPLTPEQFRYNNEDVIHAPYLAHQGWYDITKAFDGKDNLLCGAATAGNMLHWWFDQNKTEIEAYLSKHPEKQKIIFNNQELFDLKAAIDTKDSQTNSQLFNYFRDKAFPNLSARQLGVMPDLVLDMFINGYYLNVFKTQSTDVNRPYQDKDKRGGIFDAVFTRGDQTTLLTARHDLKNKGLNDISTIIKQELTEGRALALSHTYANVSISHVINLWGADFNAEGNLEAIYVTDSDANASIGMKKYFVGINAHKHVAISAKKIEGENIGAQVLGLFTLSSGKDIWQKLS

SEQ ID NO: 78 - protein, 300 aa, Artificial Sequence
  WT_del15
PHQITSVWTKGVTPLTPEQFRYNNEDVIHAPYLAHQGWYDITKAFDGKDNLLCGAATAGNMLHWWFDQNKTEIEAYLSKHPEKQKIIFNNQELFDLKAAIDTKDSQTNSQLFNYFRDKAFPNLSARQLGVMPDLVLDMFINGYYLNVFKTQSTDVNRPYQDKDKRGGIFDAVFTRGDQTTLLTARHDLKNKGLNDISTIIKQELTEGRALALSHTYANVSISHVINLWGADFNAEGNLEAIYVTDSDANASIGMKKYFVGINAHRHVAISAKKIEGENIGAQVLGLFTLSSGKDIWQKLS

SEQ ID NO: 79 - protein, 299 aa, Artificial Sequence
  WT_del16
HQITSVWTKGVTPLTPEQFRYNNEDVIHAPYLAHQGWYDITKAFDGKDNLLCGAATAGNMLHWWFDQNKTEIEAYLSKHPEKQKIIFNNQELFDLKAAIDTKDSQTNSQLFNYFRDKAFPNLSARQLGVMPDLVLDMFINGYYLNVFKTQSTDVNRPYQDKDKRGGIFDAVFTRGDQTTLLTARHDLKNKGLNDISTIIKQELTEGRALALSHTYANVSISHVINLWGADFNAEGNLEAIYVTDSDANASIGMKKYFVGINAHRHVAISAKKIEGENIGAQVLGLFTLSSGKDIWQKLS

SEQ ID NO: 80 - protein, 298 aa, Artificial Sequence
  WT_del17
QITSVWTKGVTPLTPEQFRYNNEDVIHAPYLAHQGWYDITKAFDGKDNLLCGAATAGNMLHWWFDQNKTEIEAYLSKHPEKQKIIFNNQELFDLKAAIDTKDSQTNSQLFNYFRDKAFPNLSARQLGVMPDLVLDMFINGYYLNVFKTQSTDVNRPYQDKDKRGGIFDAVFTRGDQTTLLTARHDLKNKGLNDISTIIKQELTEGRALALSHTYANVSISHVINLWGADFNAEGNLEAIYVTDSDANASIGMKKYFVGINAHRHVAISAKKIEGENIGAQVLGLFTLSSGKDIWQKLS

SEQ ID NO: 81 - protein, 297 aa, Artificial Sequence
  WT_del18
ITSVWTKGVTPLTPEQFRYNNEDVIHAPYLAHQGWYDITKAFDGKDNLLCGAATAGNMLHWWFDQNKTEIEAYLSKHPEKQKIIFNNQELFDLKAAIDTKDSQTNSQLFNYFRDKAFPNLSARQLGVMPDLVLDMFINGYYLNVFKTQSTDVNRPYQDKDKRGGIFDAVFTRGDQTTLLTARHDLKNKGLNDISTIIKQELTEGRALALSHTYANVSISHVINLWGADFNAEGNLEAIYVTDSDANASIGMKKYFVGINAHRHVAISAKKIEGENIGAQVLGLFTLSSGKDIWQKLS

SEQ ID NO: 82 - protein, 296 aa, Artificial Sequence
  WT_del19
TSVWTKGVTPLTPEQFRYNNEDVIHAPYLAHQGWYDITKAFDGKDNLLCGAATAGNMLHWWFDQNKTEIEAYLSKHPEKQKIIFNNQELFDLKAAIDTKDSQTNSQLFNYFRDKAFPNLSARQLGVMPDLVLDMFINGYYLNVFKTQSTDVNRPYQDKDKRGGIFDAVFTRGDQTTLLTARHDLKNKGLNDISTIIKQELTEGRALALSHTYANVSISHVINLWGADFNAEGNLEAIYVTDSDANASIGMKKYFVGINAHRHVAISAKKIEGENIGAQVLGLFTLSSGKDIWQKLS

SEQ ID NO: 83 - protein, 310 aa, Artificial Sequence
  WT_delC5
DDYQRNATEAYAKEVPHQITSVWTKGVTPLTPEQFRYNNEDVIHAPYLAHQGWYDITKAFDGKDNLLCGAATAGNMLHWWFDQNKTEIEAYLSKHPEKQKIIFNNQELFDLKAAIDTKDSQTNSQLFNYFRDKAFPNLSARQLGVMPDLVLDMFINGYYLNVFKTQSTDVNRPYQDKDKRGGIFDAVFTRGDQTTLLTARHDLKNKGLNDISTIIKQELTEGRALALSHTYANVSISHVINLWGADFNAEGNLEAIYVTDSDANASIGMKKYFVGINAHRHVAISAKKIEGENIGAQVLGLFTLSSGKDI

SEQ ID NO: 84 - protein, 305 aa, Artificial Sequence
  WT_delC10
DDYQRNATEAYAKEVPHQITSVWTKGVTPLTPEQFRYNNEDVIHAPYLAHQGWYDITKAFDGKDNLLCGAATAGNMLHWWFDQNKTEIEAYLSKHPEKQKIIFNNQELFDLKAAIDTKDSQTNSQLFNYFRDKAFPNLSARQLGVMPDLVLDMFINGYYLNVFKTQSTDVNRPYQDKDKRGGIFDAVFTRGDQTTLLTARHDLKNKGLNDISTIIKQELTEGRALALSHTYANVSISHVINLWGADFNAEGNLEAIYVTDSDANASIGMKKYFVGINAHRHVAISAKKIEGENIGAQVLGLFTLS

SEQ ID NO: 85 - protein, 297 aa, Artificial Sequence
  T24A_del18
ITSVWAKGVTPLTPEQFRYNNEDVIHAPYLAHQGWYDITKAFDGKDNLLCGAATAGNMLHWWFDQNKTEIEAYLSKHPEKQKIIFNNQELFDLKAAIDTKDSQTNSQLFNYFRDKAFPNLSARQLGVMPDLVLDMFINGYYLNVFKTQSTDVNRPYQDKDKRGGIFDAVFTRGDQTTLLTARHDLKNKGLNDISTIIKQELTEGRALALSHTYANVSISHVINLWGADFNAEGNLEAIYVTDSDANASIGMKKYFVGINAHRHVAISAKKIEGENIGAQVLGLFTLSSGKDIWQKLS

SEQ ID NO: 86 - protein, 297 aa, Artificial Sequence
  A59L_del18
ITSVWTKGVTPLTPEQFRYNNEDVIHAPYLAHQGWYDITKLFDGKDNLLCGAATAGNMLHWWFDQNKTEIEAYLSKHPEKQKIIFNNQELFDLKAAIDTKDSQTNSQLFNYFRDKAFPNLSARQLGVMPDLVLDMFINGYYLNVFKTQSTDVNRPYQDKDKRGGIFDAVFTRGDQTTLLTARHDLKNKGLNDISTIIKQELTEGRALALSHTYANVSISHVINLWGADFNAEGNLEAIYVTDSDANASIGMKKYFVGINAHRHVAISAKKIEGENIGAQVLGLFTLSSGKDIWQKLS

SEQ ID NO: 87 - protein, 297 aa, Artificial Sequence
  A59V_del18
ITSVWTKGVTPLTPEQFRYNNEDVIHAPYLAHQGWYDITKVFDGKDNLLCGAATAGNMLHWWFDQNKTEIEAYLSKHPEKQKIIFNNQELFDLKAAIDTKDSQTNSQLFNYFRDKAFPNLSARQLGVMPDLVLDMFINGYYLNVFKTQSTDVNRPYQDKDKRGGIFDAVFTRGDQTTLLTARHDLKNKGLNDISTIIKQELTEGRALALSHTYANVSISHVINLWGADFNAEGNLEAIYVTDSDANASIGMKKYFVGINAHRHVAISAKKIEGENIGAQVLGLFTLSSGKDIWQKLS

SEQ ID NO: 88 - protein, 297 aa, Artificial Sequence
  E97D_del18
ITSVWTKGVTPLTPEQFRYNNEDVIHAPYLAHQGWYDITKAFDGKDNLLCGAATAGNMLHWWFDQNKTEIEAYLSKHPDKQKIIFNNQELFDLKAAIDTKDSQTNSQLFNYFRDKAFPNLSARQLGVMPDLVLDMFINGYYLNVFKTQSTDVNRPYQDKDKRGGIFDAVFTRGDQTTLLTARHDLKNKGLNDISTIIKQELTEGRALALSHTYANVSISHVINLWGADFNAEGNLEAIYVTDSDANASIGMKKYFVGINAHRHVAISAKKIEGENIGAQVLGLFTLSSGKDIWQKLS

SEQ ID NO: 89 - protein, 297 aa, Artificial Sequence
  R280H_del18
ITSVWTKGVTPLTPEQFRYNNEDVIHAPYLAHQGWYDITKAFDGKDNLLCGAATAGNMLHWWFDQNKTEIEAYLSKHPEKQKIIFNNQELFDLKAAIDTKDSQTNSQLFNYFRDKAFPNLSARQLGVMPDLVLDMFINGYYLNVFKTQSTDVNRPYQDKDKRGGIFDAVFTRGDQTTLLTARHDLKNKGLNDISTIIKQELTEGRALALSHTYANVSISHVINLWGADFNAEGNLEAIYVTDSDANASIGMKKYFVGINAHHHVAISAKKIEGENIGAQVLGLFTLSSGKDIWQKLS

SEQ ID NO: 90 - protein, 292 aa, Artificial Sequence
  E97D_del18_delC5
ITSVWTKGVTPLTPEQFRYNNEDVIHAPYLAHQGWYDITKAFDGKDNLLCGAATAGNMLHWWFDQNKTEIEAYLSKHPDKQKIIFNNQELFDLKAAIDTKDSQTNSQLFNYFRDKAFPNLSARQLGVMPDLVLDMFINGYYLNVFKTQSTDVNRPYQDKDKRGGIFDAVFTRGDQTTLLTARHDLKNKGLNDISTIIKQELTEGRALALSHTYANVSISHVINLWGADFNAEGNLEAIYVTDSDANASIGMKKYFVGINAHRHVAISAKKIEGENIGAQVLGLFTLSSGKDI

SEQ ID NO: 91 - protein, 287 aa, Artificial Sequence
  E97D_del18_delC10
ITSVWTKGVTPLTPEQFRYNNEDVIHAPYLAHQGWYDITKAFDGKDNLLCGAATAGNMLHWWFDQNKTEIEAYLSKHPDKQKIIFNNQELFDLKAAIDTKDSQTNSQLFNYFRDKAFPNLSARQLGVMPDLVLDMFINGYYLNVFKTQSTDVNRPYQDKDKRGGIFDAVFTRGDQTTLLTARHDLKNKGLNDISTIIKQELTEGRALALSHTYANVSISHVINLWGADFNAEGNLEAIYVTDSDANASIGMKKYFVGINAHRHVAISAKKIEGENIGAQVLGLFTLS

SEQ ID NO: 92 - protein, 292 aa, Artificial Sequence
  A59V_del18_delC5
ITSVWTKGVTPLTPEQFRYNNEDVIHAPYLAHQGWYDITKVFDGKDNLLCGAATAGNMLHWWFDQNKTEIEAYLSKHPEKQKIIFNNQELFDLKAAIDTKDSQTNSQLFNYFRDKAFPNLSARQLGVMPDLVLDMFINGYYLNVFKTQSTDVNRPYQDKDKRGGIFDAVFTRGDQTTLLTARHDLKNKGLNDISTIIKQELTEGRALALSHTYANVSISHVINLWGADFNAEGNLEAIYVTDSDANASIGMKKYFVGINAHRHVAISAKKIEGENIGAQVLGLFTLSSGKDI

SEQ ID NO: 93 - protein, 292 aa, Artificial Sequence
  A59L_del18_delC5
ITSVWTKGVTPLTPEQFRYNNEDVIHAPYLAHQGWYDITKLFDGKDNLLCGAATAGNMLHWWFDQNKTEIEAYLSKHPEKQKIIFNNQELFDLKAAIDTKDSQTNSQLFNYFRDKAFPNLSARQLGVMPDLVLDMFINGYYLNVFKTQSTDVNRPYQDKDKRGGIFDAVFTRGDQTTLLTARHDLKNKGLNDISTIIKQELTEGRALALSHTYANVSISHVINLWGADFNAEGNLEAIYVTDSDANASIGMKKYFVGINAHRHVAISAKKIEGENIGAQVLGLFTLSSGKDI

SEQ ID NO: 94 - protein, 292 aa, Artificial Sequence
  R280H_del18_delC5
ITSVWTKGVTPLTPEQFRYNNEDVIHAPYLAHQGWYDITKAFDGKDNLLCGAATAGNMLHWWFDQNKTEIEAYLSKHPEKQKIIFNNQELFDLKAAIDTKDSQTNSQLFNYFRDKAFPNLSARQLGVMPDLVLDMFINGYYLNVFKTQSTDVNRPYQDKDKRGGIFDAVFTRGDQTTLLTARHDLKNKGLNDISTIIKQELTEGRALALSHTYANVSISHVINLWGADFNAEGNLEAIYVTDSDANASIGMKKYFVGINAHHHVAISAKKIEGENIGAQVLGLFTLSSGKDI

SEQ ID NO: 95 - protein, 315 aa, Artificial Sequence
  A59V/E97D/R280H
DDYQRNATEAYAKEVPHQITSVWTKGVTPLTPEQFRYNNEDVIHAPYLAHQGWYDITKVFDGKDNLLCGAATAGNMLHWWFDQNKTEIEAYLSKHPDKQKIIFNNQELFDLKAAIDTKDSQTNSQLFNYFRDKAFPNLSARQLGVMPDLVLDMFINGYYLNVFKTQSTDVNRPYQDKDKRGGIFDAVFTRGDQTTLLTARHDLKNKGLNDISTIIKQELTEGRALALSHTYANVSISHVINLWGADFNAEGNLEAIYVTDSDANASIGMKKYFVGINAHHHVAISAKKIEGENIGAQVLGLFTLSSGKDIWQKLS